European Patent Specification EP 4 573 214 B1, published March 11, 2026. Title: NUCLEIC ACID AMPLIFICATION. Applicant: SiMSen Diagnostics AB. Application SE. The sequence listing filed with the application follows.

SEQUENCE LISTING (100 sequences)

SEQ ID NO: 1 - DNA, 70 bp, synthetic construct
  source 1..70: mol_type = other DNA
ggacactctttccctacacgacgctcttccgatctnantnancntntncntnanatgggaaagagtgtcc

SEQ ID NO: 2 - DNA, 14 bp, synthetic construct
  source 1..14: mol_type = other DNA
ggacactctttccc

SEQ ID NO: 3 - DNA, 14 bp, synthetic construct
  source 1..14: mol_type = other DNA
gggaaagagtgtcc

SEQ ID NO: 4 - DNA, 35 bp, synthetic construct
  source 1..35: mol_type = other DNA
ggacactctttccctacacgacgctcttccgatct

SEQ ID NO: 5 - DNA, 34 bp, synthetic construct
  source 1..34: mol_type = other DNA
gtgactggagttcagacgtgtgctcttccgatct

SEQ ID NO: 6 - DNA, 20 bp, synthetic construct
  source 1..20: mol_type = other DNA
aatgatacggcgaccaccga

SEQ ID NO: 7 - DNA, 29 bp, synthetic construct
  source 1..29: mol_type = other DNA
aatgatacggcgaccaccgagatctacac

SEQ ID NO: 8 - DNA, 24 bp, synthetic construct
  source 1..24: mol_type = other DNA
caagcagaagacggcatacgagat

SEQ ID NO: 9 - DNA, 63 bp, synthetic construct
  source 1..63: mol_type = other DNA
ggacactctttccctacacgacgctcttccgatctnnnnnnnnnnnnatgggaaagagtgtcc

SEQ ID NO: 10 - DNA, 34 bp, synthetic construct
  source 1..34: mol_type = other DNA
tgctcattttgaagtaaatccagattgttctgtt

SEQ ID NO: 11 - DNA, 31 bp, synthetic construct
  source 1..31: mol_type = other DNA
actgcaagtcgagaggtattcagaatacatt

SEQ ID NO: 12 - DNA, 17 bp, synthetic construct
  source 1..17: mol_type = other DNA
tgggacccactccatcg

SEQ ID NO: 13 - DNA, 28 bp, synthetic construct
  source 1..28: mol_type = other DNA
atatttcttcatgaagacctcacagtaa

SEQ ID NO: 14 - DNA, 16 bp, synthetic construct
  source 1..16: mol_type = other DNA
caactgcgccgacccc

SEQ ID NO: 15 - DNA, 18 bp, synthetic construct
  source 1..18: mol_type = other DNA
cagcgtgtccaggaagcc

SEQ ID NO: 16 - DNA, 20 bp, synthetic construct
  source 1..20: mol_type = other DNA
ttgcacactgtcagcaaaac

SEQ ID NO: 17 - DNA, 21 bp, synthetic construct
  source 1..21: mol_type = other DNA
accaataactccaaggctggt

SEQ ID NO: 18 - DNA, 26 bp, synthetic construct
  source 1..26: mol_type = other DNA
gtcactggcagcaacagtcttacctg

SEQ ID NO: 19 - DNA, 28 bp, synthetic construct
  source 1..28: mol_type = other DNA
ttcctcaggattgcctttaccactcaga

SEQ ID NO: 20 - DNA, 24 bp, synthetic construct
  source 1..24: mol_type = other DNA
tggcctgcaggattatgtcttatt

SEQ ID NO: 21 - DNA, 22 bp, synthetic construct
  source 1..22: mol_type = other DNA
ccaggaaacgcacaacactcag

SEQ ID NO: 22 - DNA, 23 bp, synthetic construct
  source 1..23: mol_type = other DNA
ctgaatacaggttatcagtgcct

SEQ ID NO: 23 - DNA, 27 bp, synthetic construct
  source 1..27: mol_type = other DNA
tcaaagatcctgtgcagaaaaatgaat

SEQ ID NO: 24 - DNA, 25 bp, synthetic construct
  source 1..25: mol_type = other DNA
tgcagagttcagttaccttaggaga

SEQ ID NO: 25 - DNA, 22 bp, synthetic construct
  source 1..22: mol_type = other DNA
tgcatacatcagacagcacaga

SEQ ID NO: 26 - DNA, 23 bp, synthetic construct
  source 1..23: mol_type = other DNA
ccatgacaagattttcccttacc

SEQ ID NO: 27 - DNA, 25 bp, synthetic construct
  source 1..25: mol_type = other DNA
caccttatatgggcatacttccact

SEQ ID NO: 28 - DNA, 18 bp, synthetic construct
  source 1..18: mol_type = other DNA
ccaccttgggctacctgc

SEQ ID NO: 29 - DNA, 20 bp, synthetic construct
  source 1..20: mol_type = other DNA
ggtactcgatgatgccggtg

SEQ ID NO: 30 - DNA, 23 bp, synthetic construct
  source 1..23: mol_type = other DNA
gtcctttcaggatggtggatgtg

SEQ ID NO: 31 - DNA, 23 bp, synthetic construct
  source 1..23: mol_type = other DNA
ggatgtcacgttctcaaagcagt

SEQ ID NO: 32 - DNA, 21 bp, synthetic construct
  source 1..21: mol_type = other DNA
attcgatgatccctgtggtgg

SEQ ID NO: 33 - DNA, 20 bp, synthetic construct
  source 1..20: mol_type = other DNA
gtagctgaccctgcctacct

SEQ ID NO: 34 - DNA, 25 bp, synthetic construct
  source 1..25: mol_type = other DNA
gcagtgtatccattttcttctctct

SEQ ID NO: 35 - DNA, 25 bp, synthetic construct
  source 1..25: mol_type = other DNA
gtattgttaaccttgcagaatggtc

SEQ ID NO: 36 - DNA, 21 bp, synthetic construct
  source 1..21: mol_type = other DNA
gcgatgacggaatataagctg

SEQ ID NO: 37 - DNA, 20 bp, synthetic construct
  source 1..20: mol_type = other DNA
ctggatcagctggatggtca

SEQ ID NO: 38 - DNA, 27 bp, synthetic construct
  source 1..27: mol_type = other DNA
ccaacatgacttacttgatccccataa

SEQ ID NO: 39 - DNA, 25 bp, synthetic construct
  source 1..25: mol_type = other DNA
cttgtgagtggatgggtaaaaccta

SEQ ID NO: 40 - DNA, 19 bp, synthetic construct
  source 1..19: mol_type = other DNA
agtggatcccctctccacc

SEQ ID NO: 41 - DNA, 20 bp, synthetic construct
  source 1..20: mol_type = other DNA
tagtccctggctggaccaag

SEQ ID NO: 42 - DNA, 18 bp, synthetic construct
  source 1..18: mol_type = other DNA
agggagctgcaggttctg

SEQ ID NO: 43 - DNA, 19 bp, synthetic construct
  source 1..19: mol_type = other DNA
gccatcgctgtagaacgca

SEQ ID NO: 44 - DNA, 20 bp, synthetic construct
  source 1..20: mol_type = other DNA
gcagatgtcaagccctccaa

SEQ ID NO: 45 - DNA, 20 bp, synthetic construct
  source 1..20: mol_type = other DNA
gctgaccccaaagtcacaga

SEQ ID NO: 46 - DNA, 20 bp, synthetic construct
  source 1..20: mol_type = other DNA
cgccttgaggcctttcttac

SEQ ID NO: 47 - DNA, 21 bp, synthetic construct
  source 1..21: mol_type = other DNA
gtcgtcatccttcagttctcc

SEQ ID NO: 48 - DNA, 25 bp, synthetic construct
  source 1..25: mol_type = other DNA
aacctctctttcttccacctttctc

SEQ ID NO: 49 - DNA, 24 bp, synthetic construct
  source 1..24: mol_type = other DNA
cttatgatctggttccggattgcg

SEQ ID NO: 50 - DNA, 27 bp, synthetic construct
  source 1..27: mol_type = other DNA
tcatcagttcctcctcagaattccccc

SEQ ID NO: 51 - DNA, 29 bp, synthetic construct
  source 1..29: mol_type = other DNA
aagcatacctggtataaacagtggcacac

SEQ ID NO: 52 - DNA, 24 bp, synthetic construct
  source 1..24: mol_type = other DNA
gctggattgtcagtgcgcttttcc

SEQ ID NO: 53 - DNA, 27 bp, synthetic construct
  source 1..27: mol_type = other DNA
gactgagtacaaactggtggtggttgg

SEQ ID NO: 54 - DNA, 20 bp, synthetic construct
  source 1..20: mol_type = other DNA
cgcatttaccccaagggagg

SEQ ID NO: 55 - DNA, 21 bp, synthetic construct
  source 1..21: mol_type = other DNA
cagccagcgttccagaaaatc

SEQ ID NO: 56 - DNA, 21 bp, synthetic construct
  source 1..21: mol_type = other DNA
agccttcgtgcactagttgat

SEQ ID NO: 57 - DNA, 25 bp, synthetic construct
  source 1..25: mol_type = other DNA
gtgcctttctaaattgcagtttgtt

SEQ ID NO: 58 - DNA, 31 bp, synthetic construct
  source 1..31: mol_type = other DNA
acttgcctactgatcagttacacaaccaatg

SEQ ID NO: 59 - DNA, 36 bp, synthetic construct
  source 1..36: mol_type = other DNA
ggttaattcccaatttaagatacttacacagtaggg

SEQ ID NO: 60 - DNA, 21 bp, synthetic construct
  source 1..21: mol_type = other DNA
ggctcccataactgcctgaat

SEQ ID NO: 61 - DNA, 23 bp, synthetic construct
  source 1..23: mol_type = other DNA
ggatttggttgtgaagattcgct

SEQ ID NO: 62 - DNA, 24 bp, synthetic construct
  source 1..24: mol_type = other DNA
ccatgtaagtcctagcattcattt

SEQ ID NO: 63 - DNA, 23 bp, synthetic construct
  source 1..23: mol_type = other DNA
tgtactctttttcctgttgctgt

SEQ ID NO: 64 - DNA, 22 bp, synthetic construct
  source 1..22: mol_type = other DNA
gaggctacaacagcaaaagctc

SEQ ID NO: 65 - DNA, 25 bp, synthetic construct
  source 1..25: mol_type = other DNA
ctatgatctctaccatgagacctga

SEQ ID NO: 66 - DNA, 21 bp, synthetic construct
  source 1..21: mol_type = other DNA
agatggcacagcccataagaa

SEQ ID NO: 67 - DNA, 19 bp, synthetic construct
  source 1..19: mol_type = other DNA
gaagtcctggcaagcgaga

SEQ ID NO: 68 - DNA, 20 bp, synthetic construct
  source 1..20: mol_type = other DNA
gcaatggccaaagcactgat

SEQ ID NO: 69 - DNA, 23 bp, synthetic construct
  source 1..23: mol_type = other DNA
cctgtgtttggttttgtaggtct

SEQ ID NO: 70 - DNA, 25 bp, synthetic construct
  source 1..25: mol_type = other DNA
accatcaatcagttgttcttcaagt

SEQ ID NO: 71 - DNA, 23 bp, synthetic construct
  source 1..23: mol_type = other DNA
aaatggtgatggagacaattgag

SEQ ID NO: 72 - DNA, 21 bp, synthetic construct
  source 1..21: mol_type = other DNA
gtacgtcactgctctgcgccg

SEQ ID NO: 73 - DNA, 28 bp, synthetic construct
  source 1..28: mol_type = other DNA
ggtaggaatggagggaagagaacctgaa

SEQ ID NO: 74 - DNA, 18 bp, synthetic construct
  source 1..18: mol_type = other DNA
gtggcaagtggctcctga

SEQ ID NO: 75 - DNA, 16 bp, synthetic construct
  source 1..16: mol_type = other DNA
catgggcggcatgaac

SEQ ID NO: 76 - DNA, 19 bp, synthetic construct
  source 1..19: mol_type = other DNA
ggcccctgtcatcttctgt

SEQ ID NO: 77 - DNA, 20 bp, synthetic construct
  source 1..20: mol_type = other DNA
cagaatgcaagaagcccaga

SEQ ID NO: 78 - DNA, 20 bp, synthetic construct
  source 1..20: mol_type = other DNA
ttgcgtgtggagtatttgga

SEQ ID NO: 79 - DNA, 20 bp, synthetic construct
  source 1..20: mol_type = other DNA
agacctcaggcggctcatag

SEQ ID NO: 80 - DNA, 27 bp, synthetic construct
  source 1..27: mol_type = other DNA
cttccagtgtgatgatggtgaggatgg

SEQ ID NO: 81 - DNA, 26 bp, synthetic construct
  source 1..26: mol_type = other DNA
acatgtgtaacagttcctgcatgggc

SEQ ID NO: 82 - DNA, 20 bp, synthetic construct
  source 1..20: mol_type = other DNA
tcctctgttgctgcagatcc

SEQ ID NO: 83 - DNA, 20 bp, synthetic construct
  source 1..20: mol_type = other DNA
tgagttccaaggcctcattc

SEQ ID NO: 84 - DNA, 22 bp, synthetic construct
  source 1..22: mol_type = other DNA
cctggtgtgggtcttcaggtgg

SEQ ID NO: 85 - DNA, 32 bp, synthetic construct
  source 1..32: mol_type = other DNA
gtgtgaaaccattccagtgtaaaacttgtcag

SEQ ID NO: 86 - DNA, 18 bp, synthetic construct
  source 1..18: mol_type = other DNA
gtggcaagtggctcctga

SEQ ID NO: 87 - DNA, 16 bp, synthetic construct
  source 1..16: mol_type = other DNA
catgggcggcatgaac

SEQ ID NO: 88 - DNA, 14 bp, synthetic construct
  source 1..14: mol_type = other DNA
sswswwwswwswss

SEQ ID NO: 89 - DNA, 21 bp, synthetic construct
  source 1..21: mol_type = other DNA
swsswwwsswswwwswwswss

SEQ ID NO: 90 - DNA, 23 bp, synthetic construct
  source 1..23: mol_type = other DNA
nantnancntntncntnantnan

SEQ ID NO: 91 - DNA, 73 bp, synthetic construct
  source 1..73: mol_type = other DNA
ggacactctttccctacacgacgctcttccgatctatgggaaagagtgtcccttacctgaggagacggtgacc

SEQ ID NO: 92 - DNA, 59 bp, synthetic construct
  source 1..59: mol_type = other DNA
gtgactggagttcagacgtgtgctcttccgatcttggagctgagcagcctgagatctga

SEQ ID NO: 93 - DNA, 59 bp, synthetic construct
  source 1..59: mol_type = other DNA
gtgactggagttcagacgtgtgctcttccgatctcaatgaccaacatggaccctgtgga

SEQ ID NO: 94 - DNA, 59 bp, synthetic construct
  source 1..59: mol_type = other DNA
gtgactggagttcagacgtgtgctcttccgatcttctgcaaatgaacagcctgagagcc

SEQ ID NO: 95 - DNA, 59 bp, synthetic construct
  source 1..59: mol_type = other DNA
gtgactggagttcagacgtgtgctcttccgatctgagctctgtgaccgccgcggacacg

SEQ ID NO: 96 - DNA, 59 bp, synthetic construct
  source 1..59: mol_type = other DNA
gtgactggagttcagacgtgtgctcttccgatctcagcaccgcctacctgcagtggagc

SEQ ID NO: 97 - DNA, 59 bp, synthetic construct
  source 1..59: mol_type = other DNA
gtgactggagttcagacgtgtgctcttccgatctgttctccctgcagctgaactctgtg

SEQ ID NO: 98 - DNA, 58 bp, synthetic construct
  source 1..58: mol_type = other DNA
gtgactggagttcagacgtgtgctcttccgatctcagcacggcatatctgcagatcag

SEQ ID NO: 99 - DNA, 35 bp, synthetic construct
  source 1..35: mol_type = other DNA
nantnancntntncntnanatgggaaagagtgtcc

SEQ ID NO: 100 - DNA, 33 bp, synthetic construct
  source 1..33: mol_type = other DNA
acactctttccctacacgacgctcttccgatct